European Patent Specification EP 3 966 351 B1, published April 29, 2026. Title: COMPOSITIONS AND METHODS FOR DETECTION OF NEISSERIA GONORROHEAE. Applicant: F. Hoffmann-La Roche AG Roche Diagnostics GmbH Roche Molecular Systems, Inc. The sequence listing filed with the application follows.

SEQUENCE LISTING (5 sequences)

SEQ ID NO: 1 - DNA, 14 bp, Artificial Sequence
  R6_1483F_TBBC forward primer
  modified_base (14)..(14): t-butyl-benzyl dC
cgcagcatacgcgc

SEQ ID NO: 2 - DNA, 20 bp, Artificial Sequence
  R6_1483R_TBB reverse primer
  modified_base (20)..(20): t-butyl-benzyl dC
atggctttgatgatttgcgc

SEQ ID NO: 3 - DNA, 29 bp, Artificial Sequence
  R6_1483_P probe
  misc_feature: 5` HEX
  misc_feature: 3` phosphate
  misc_feature (5)..(6): BHQ-2
tcatcacgcggcaaaagatgaagaagcgg

SEQ ID NO: 4 - DNA, 975 bp, Neisseria gonorrhoeae
ttacgccgatttgtaacgcgatggatcgtaatctccgcctttcttatgtacgtgatacgcaataacggcgagtttacgcatcaatgctgcgatgatgacttttttaggcttcttcttttcttccagccttttgatgaagtcgggaaatgcccttatccggtatgcgaccatggccggcataaacaagacggcgcgtaatttcctgttgccaaacttggtcagtttgccttttccccttacgcttgtcccggattctttttgttgcgggcttaagcctgcgaacgctgcaaatttgtttgatgtttcaaatttcgaagatgttagatgatgaaacaatacggctgcggtcattctgcctattgccggtatggtttcaagacgcttcacgccttccttgcagttaggcttctccgtctgctcttttatcttctcctttaaaacttcaagctgttcattcatggctttgatgatttgcgcatatgctttggccgcttcttcatcttttgccgcgtgatgacggtttttcattgccgcgcattcgcttttgatttgcgcgtatgctgcggtcatccgtaaaagcctgtattgctcgtccgtaggcttctgcctctttacaagctcgctttctttcgccaaccggcaatactgcgctatcagctttgcatcctgtttgtctgttttggttcgcttgaacctgctttctgcatacttgcttattttcagcggattcactacgtaaacgctgtaatactgcgcgaagtagtcggcaacttcttcataatagtttcccgttgcctccatgcagatatgcagattctgacatcccaagcttttcaaccggtccgaaaactgatctaaaccttttgaatcgttgtcaaactttgccgaatgctccgttttgccgaccatggcggatgcgttaaaggtcagtttcgatatatccaatcctacggcgttacgcatgggattaccctt

SEQ ID NO: 5 - DNA, 806 bp, Neisseria gonorrhoeae
cagccgcatcatgatgccgcacgtcagggcttcgtcttccgatacctttgcgccagacaacatccgggcgatgttttctttttgcgcttttgaccgggcggacagccggttccggtcaacgtttctgaccgtcccggcgcgtttgacggcgcgttcctgccgcgttgattccttcgccgcgcgtttggcggcaagcatctgttttgccgtcggttttgttgctactgtttgcattttgttttctcgattttttgatgccgttctctcaatgcccaatcataaagctgtatctctcacgaggtcgccgaatttaaattgatagttcatgtcttgttccattaatatcaaacgcaatcttcaaacacctcaattacattttttaaatcgctaataccataatttattacatcctttagaaattccaaagaggtatccgcttcgtctgctttatccctaatttcgtctatataaccctctaacgattcaggctcttttaatgcttctttgcataagttatctattacccttaatgcgttttttacatcttccaaatagctcattttttgctccttaactcaaaatgggatgctgtcgtcaacatcttctacggtttatctaatctgcaaattcttccgcccttcaatcttcgcgcctgctacttgccgaccgctttcaatcgcttttctgatggcggttttgtccggttcggttttgacggcctcacgcataaattcggcggggatttgtgcttcgtctaagatcacgacggcttcggatttgcggaacgaggctttaaaagtgccgtc